European Patent Application EP 4 488 378 A1, published January 8, 2025. Title: METHOD FOR PRODUCING FC-CONTAINING MOLECULE. Applicant: DAIICHI SANKYO COMPANY, LIMITED. Application EP 23763495.1, filed March 1, 2023. The sequence listing filed with the application follows.

SEQUENCE LISTING (81 sequences)

SEQ ID NO: 1 - protein, 218 aa, synthetic construct
  REGION 1..218: note = Anti-CD70 Antibody 1 Light Chain
DIVMTQSPDSLAVSLGERATINCRASKSVSTSGYSFMHWYQQKPGQPPKLLIYLASNLESGVPDRFSGSGSGTDFTLTISSLQAEDVAVYYCQHSREVPWTFGQGTKVEIKRTVAAPSVFIFPPSDEQLKSGTASVVCLLNNFYPREAKVQWKVDNALQSGNSQESVTEQDSKDSTYSLSSTLTLSKADYEKHKVYACEVTHQGLSSPVTKSFNRGEC

SEQ ID NO: 2 - protein, 448 aa, synthetic construct
  REGION 1..448: note = Anti-CD70 Antibody 1 Heavy Chain
QVQLVQSGAEVKKPGASVKVSCKASGYTFTNYGMNWVRQAPGQGLKWMGWINTYTGEPTYADAFKGRVTMTRDTSISTAYMELSRLRSDDTAVYYCARDYGDYGMDYWGQGTTVTVSSASTKGPSVFPLAPSSKSTSGGTAALGCLVKDYFPEPVTVSWNSGALTSGVHTFPAVLQSSGLYSLSSVVTVPSSSLGTQTYICNVNHKPSNTKVDKRVEPKSCDKTHTCPPCPAPEAAGGPSVFLFPPKPKDTLMISRTPEVTCVVVDVSHEDPEVKFNWYVDGVEVHNAKTKPREEQYNSTYRVVSVLTVLHQDWLNGKEYKCKVSNKALPAPIEKTISKAKGQPREPQVYTLPPSREEMTKNQVSLTCLVKGFYPSDIAVEWESNGQPENNYKTTPPVLDSDGSFFLYSKLTVDKSRWQQGNVFSCSVMHEALHNHYTQKSLSLSPGK

SEQ ID NO: 3 - protein, 214 aa, synthetic construct
  REGION 1..214: note = Anti-CD70 Antibody 2 Light Chain
EIVLTQSPATLSLSPGERATLSCRASQSVSSYLAWYQQKPGQAPRLLIYDASNRATGIPARFSGSGSGTDFTLTISSLEPEDFAVYYCQQRTNWPLTFGGGTKVEIKRTVAAPSVFIFPPSDEQLKSGTASVVCLLNNFYPREAKVQWKVDNALQSGNSQESVTEQDSKDSTYSLSSTLTLSKADYEKHKVYACEVTHQGLSSPVTKSFNRGEC

SEQ ID NO: 4 - protein, 448 aa, synthetic construct
  REGION 1..448: note = Anti-CD70 Antibody 2 Heavy Chain
QVQLVESGGGVVQPGRSLRLSCAASGFTFSSYIMHWVRQAPGKGLEWVAVISYDGRNKYYADSVKGRFTISRDNSKNTLYLQMNSLRAEDTAVYYCARDTDGYDFDYWGQGTLVTVSSASTKGPSVFPLAPSSKSTSGGTAALGCLVKDYFPEPVTVSWNSGALTSGVHTFPAVLQSSGLYSLSSVVTVPSSSLGTQTYICNVNHKPSNTKVDKRVEPKSCDKTHTCPPCPAPEAAGGPSVFLFPPKPKDTLMISRTPEVTCVVVDVSHEDPEVKFNWYVDGVEVHNAKTKPREEQYNSTYRVVSVLTVLHQDWLNGKEYKCKVSNKALPAPIEKTISKAKGQPREPQVYTLPPSREEMTKNQVSLTCLVKGFYPSDIAVEWESNGQPENNYKTTPPVLDSDGSFFLYSKLTVDKSRWQQGNVFSCSVMHEALHNHYTQKSLSLSPGK

SEQ ID NO: 5 - protein, 214 aa, synthetic construct
  REGION 1..214: note = Anti-TROP2 Antibody 1 Light Chain
DIQMTQSPSSLSASVGDRVTITCKASQDVSTAVAWYQQKPGKAPKLLIYSASYRYTGVPSRFSGSGSGTDFTLTISSLQPEDFAVYYCQQHYITPLTFGQGTKLEIKRTVAAPSVFIFPPSDEQLKSGTASVVCLLNNFYPREAKVQWKVDNALQSGNSQESVTEQDSKDSTYSLSSTLTLSKADYEKHKVYACEVTHQGLSSPVTKSFNRGEC

SEQ ID NO: 6 - protein, 451 aa, synthetic construct
  REGION 1..451: note = Anti-TROP2 Antibody 1 Heavy Chain
QVQLVQSGAEVKKPGASVKVSCKASGYTFTTAGMQWVRQAPGQGLEWMGWINTHSGVPKYAEDFKGRVTISADTSTSTAYLQLSSLKSEDTAVYYCARSGFGSSYWYFDVWGQGTLVTVSSASTKGPSVFPLAPSSKSTSGGTAALGCLVKDYFPEPVTVSWNSGALTSGVHTFPAVLQSSGLYSLSSVVTVPSSSLGTQTYICNVNHKPSNTKVDKRVEPKSCDKTHTCPPCPAPELLGGPSVFLFPPKPKDTLMISRTPEVTCVVVDVSHEDPEVKFNWYVDGVEVHNAKTKPREEQYNSTYRVVSVLTVLHQDWLNGKEYKCKVSNKALPAPIEKTISKAKGQPREPQVYTLPPSREEMTKNQVSLTCLVKGFYPSDIAVEWESNGQPENNYKTTPPVLDSDGSFFLYSKLTVDKSRWQQGNVFSCSVMHEALHNHYTQKSLSLSPGK

SEQ ID NO: 7 - protein, 214 aa, synthetic construct; identical to SEQ ID NO: 5
  REGION 1..214: note = Anti-TROP2 Antibody 2 Light Chain

SEQ ID NO: 8 - protein, 451 aa, synthetic construct
  REGION 1..451: note = Anti-TROP2 Antibody 2 Heavy Chain
QVQLVQSGAEVKKPGASVKVSCKASGYTFTTAGMQWVRQAPGQGLEWMGWINTHSGVPKYAEDFKGRVTISADTSTSTAYLQLSSLKSEDTAVYYCARSGFGSSYWYFDVWGQGTLVTVSSASTKGPSVFPLAPSSKSTSGGTAALGCLVKDYFPEPVTVSWNSGALTSGVHTFPAVLQSSGLYSLSSVVTVPSSSLGTQTYICNVNHKPSNTKVDKRVEPKSCDKTHTCPPCPAPEAAGGPSVFLFPPKPKDTLMISRTPEVTCVVVDVSHEDPEVKFNWYVDGVEVHNAKTKPREEQYNSTYRVVSVLTVLHQDWLNGKEYKCKVSNKALPAPIEKTISKAKGQPREPQVYTLPPSREEMTKNQVSLTCLVKGFYPSDIAVEWESNGQPENNYKTTPPVLDSDGSFFLYSKLTVDKSRWQQGNVFSCSVMHEALHNHYTQKSLSLSPGK

SEQ ID NO: 9 - protein, 214 aa, synthetic construct
  REGION 1..214: note = Anti-EGFR Antibody 1 Light Chain
DIQMTQSPSSLSASVGDRVTITCQASQDISNYLNWYQQKPGKAPKLLIYDASNLETGVPSRFSGSGSGTDFTFTISSLQPEDIATYFCQHFDHLPLAFGGGTKVEIKRTVAAPSVFIFPPSDEQLKSGTASVVCLLNNFYPREAKVQWKVDNALQSGNSQESVTEQDSKDSTYSLSSTLTLSKADYEKHKVYACEVTHQGLSSPVTKSFNRGEC

SEQ ID NO: 10 - protein, 449 aa, synthetic construct
  REGION 1..449: note = Anti-EGFR Antibody 1 Heavy Chain
QVQLQESGPGLVKPSETLSLTCTVSGGSVSSGDYYWTWIRQSPGKGLEWIGHIYYSGNTNYNPSLKSRLTISIDTSKTQFSLKLSSVTAADTAIYYCVRDRVTGAFDIWGQGTMVTVSSASTKGPSVFPLAPSSKSTSGGTAALGCLVKDYFPEPVTVSWNSGALTSGVHTFPAVLQSSGLYSLSSVVTVPSSSLGTQTYICNVNHKPSNTKVDKRVEPKSCDKTHTCPPCPAPEAAGGPSVFLFPPKPKDTLMISRTPEVTCVVVDVSHEDPEVKFNWYVDGVEVHNAKTKPREEQYNSTYRVVSVLTVLHQDWLNGKEYKCKVSNKALPAPIEKTISKAKGQPREPQVYTLPPSREEMTKNQVSLTCLVKGFYPSDIAVEWESNGQPENNYKTTPPVLDSDGSFFLYSKLTVDKSRWQQGNVFSCSVMHEALHNHYTQKSLSLSPGK

SEQ ID NO: 11 - protein, 214 aa, synthetic construct
  REGION 1..214: note = Anti-EGFR Antibody 2 Light Chain
DILMTQSPSSMSVSLGDTVSITCHSSQDINSNIGWLQQRPGKSFKGLIYHGTNLDDEVPSRFSGSGSGADYSLTISSLESEDFADYYCVQYAQFPWTFGGGTKLEIKRTVAAPSVFIFPPSDEQLKSGTASVVCLLNNFYPREAKVQWKVDNALQSGNSQESVTEQDSKDSTYSLSSTLTLSKADYEKHKVYACEVTHQGLSSPVTKSFNRGEC

SEQ ID NO: 12 - protein, 446 aa, synthetic construct
  REGION 1..446: note = Anti-EGFR Antibody 2 Heavy Chain
DVQLQESGPSLVKPSQSLSLTCTVTGYSITSDFAWNWIRQFPGNKLEWMGYISYSGNTRYNPSLKSRISITRDTSKNQFFLQLNSVTIEDTATYYCVTAGRGFPYWGQGTLVTVSAASTKGPSVFPLAPSSKSTSGGTAALGCLVKDYFPEPVTVSWNSGALTSGVHTFPAVLQSSGLYSLSSVVTVPSSSLGTQTYICNVNHKPSNTKVDKRVEPKSCDKTHTCPPCPAPEAAGGPSVFLFPPKPKDTLMISRTPEVTCVVVDVSHEDPEVKFNWYVDGVEVHNAKTKPREEQYNSTYRVVSVLTVLHQDWLNGKEYKCKVSNKALPAPIEKTISKAKGQPREPQVYTLPPSREEMTKNQVSLTCLVKGFYPSDIAVEWESNGQPENNYKTTPPVLDSDGSFFLYSKLTVDKSRWQQGNVFSCSVMHEALHNHYTQKSLSLSPGK

SEQ ID NO: 13 - protein, 15 aa, synthetic construct
  REGION 1..15: note = Anti-CD70 Antibody 1 CDRL1
RASKSVSTSGYSFMH

SEQ ID NO: 14 - protein, 7 aa, synthetic construct
  REGION 1..7: note = Anti-CD70 Antibody 1 CDRL2
LASNLES

SEQ ID NO: 15 - protein, 9 aa, synthetic construct
  REGION 1..9: note = Anti-CD70 Antibody 1 CDRL3
QHSREVPWT

SEQ ID NO: 16 - protein, 10 aa, synthetic construct
  REGION 1..10: note = Anti-CD70 Antibody 1 CDRH1
GYTFTNYGMN

SEQ ID NO: 17 - protein, 17 aa, synthetic construct
  REGION 1..17: note = Anti-CD70 Antibody 1 CDRH2
WINTYTGEPTYADAFKG

SEQ ID NO: 18 - protein, 9 aa, synthetic construct
  REGION 1..9: note = Anti-CD70 Antibody 1 CDRH3
DYGDYGMDY

SEQ ID NO: 19 - protein, 11 aa, synthetic construct
  REGION 1..11: note = Anti-CD70 Antibody 2 CDRL1
RASQSVSSYLA

SEQ ID NO: 20 - protein, 7 aa, synthetic construct
  REGION 1..7: note = Anti-CD70 Antibody 2 CDRL2
DASNRAT

SEQ ID NO: 21 - protein, 9 aa, synthetic construct
  REGION 1..9: note = Anti-CD70 Antibody 2 CDRL3
QQRTNWPLT

SEQ ID NO: 22 - protein, 5 aa, synthetic construct
  REGION 1..5: note = Anti-CD70 Antibody 2 CDRH1
SYIMH

SEQ ID NO: 23 - protein, 17 aa, synthetic construct
  REGION 1..17: note = Anti-CD70 Antibody 2 CDRH2
VISYDGRNKYYADSVKG

SEQ ID NO: 24 - protein, 9 aa, synthetic construct
  REGION 1..9: note = Anti-CD70 Antibody 2 CDRH3
DTDGYDFDY

SEQ ID NO: 25 - protein, 11 aa, synthetic construct
  REGION 1..11: note = Anti-TROP2 Antibody 1 CDRL1
KASQDVSTAVA

SEQ ID NO: 26 - protein, 7 aa, synthetic construct
  REGION 1..7: note = Anti-TROP2 Antibody 1 CDRL2
SASYRYT

SEQ ID NO: 27 - protein, 9 aa, synthetic construct
  REGION 1..9: note = Anti-TROP2 Antibody 1 CDRL3
QQHYITPLT

SEQ ID NO: 28 - protein, 5 aa, synthetic construct
  REGION 1..5: note = Anti-TROP2 Antibody 1 CDRH1
TAGMQ

SEQ ID NO: 29 - protein, 17 aa, synthetic construct
  REGION 1..17: note = Anti-TROP2 Antibody 1 CDRH2
WINTHSGVPKYAEDFKG

SEQ ID NO: 30 - protein, 12 aa, synthetic construct
  REGION 1..12: note = Anti-TROP2 Antibody 1 CDRH3
SGFGSSYWYFDV

SEQ ID NO: 31 - protein, 11 aa, synthetic construct
  REGION 1..11: note = Anti-TROP2 Antibody 2 CDRL1
KASQDVSTAVA

SEQ ID NO: 32 - protein, 7 aa, synthetic construct
  REGION 1..7: note = Anti-TROP2 Antibody 2 CDRL2
SASYRYT

SEQ ID NO: 33 - protein, 9 aa, synthetic construct
  REGION 1..9: note = Anti-TROP2 Antibody 2 CDRL3
QQHYITPLT

SEQ ID NO: 34 - protein, 5 aa, synthetic construct
  REGION 1..5: note = Anti-TROP2 Antibody 2 CDRH1
TAGMQ

SEQ ID NO: 35 - protein, 17 aa, synthetic construct
  REGION 1..17: note = Anti-TROP2 Antibody 2 CDRH2
WINTHSGVPKYAEDFKG

SEQ ID NO: 36 - protein, 12 aa, synthetic construct
  REGION 1..12: note = Anti-TROP2 Antibody 2 CDRH3
SGFGSSYWYFDV

SEQ ID NO: 37 - protein, 11 aa, synthetic construct
  REGION 1..11: note = Anti-EGFR Antibody 1 CDRL1
QASQDISNYLN

SEQ ID NO: 38 - protein, 7 aa, synthetic construct
  REGION 1..7: note = Anti-EGFR Antibody 1 CDRL2
DASNLET

SEQ ID NO: 39 - protein, 9 aa, synthetic construct
  REGION 1..9: note = Anti-EGFR Antibody 1 CDRL3
QHFDHLPLA

SEQ ID NO: 40 - protein, 7 aa, synthetic construct
  REGION 1..7: note = Anti-EGFR Antibody 1 CDRH1
SGDYYWT

SEQ ID NO: 41 - protein, 17 aa, synthetic construct
  REGION 1..17: note = Anti-EGFR Antibody 1 CDRH2
GHIYYSGNTNYNPSLKS

SEQ ID NO: 42 - protein, 9 aa, synthetic construct
  REGION 1..9: note = Anti-EGFR Antibody 1 CDRH3
DRVTGAFDI

SEQ ID NO: 43 - protein, 11 aa, synthetic construct
  REGION 1..11: note = Anti-EGFR Antibody 2 CDRL1
HSSQDINSNIG

SEQ ID NO: 44 - protein, 7 aa, synthetic construct
  REGION 1..7: note = Anti-EGFR Antibody 2 CDRL2
HGTNLDD

SEQ ID NO: 45 - protein, 9 aa, synthetic construct
  REGION 1..9: note = Anti-EGFR Antibody 2 CDRL3
VQYAQFPWT

SEQ ID NO: 46 - protein, 11 aa, synthetic construct
  REGION 1..11: note = Anti-EGFR Antibody 2 CDRH1
GYSITSDFAWN

SEQ ID NO: 47 - protein, 16 aa, synthetic construct
  REGION 1..16: note = Anti-EGFR Antibody 2 CDRH2
GYISYSGNTRYNPSLK

SEQ ID NO: 48 - protein, 9 aa, synthetic construct
  REGION 1..9: note = Anti-EGFR Antibody 2 CDRH3
VTAGRGFPY

SEQ ID NO: 49 - protein, 214 aa, synthetic construct
  REGION 1..214: note = Trastuzumab Light Chain
DIQMTQSPSSLSASVGDRVTITCRASQDVNTAVAWYQQKPGKAPKLLIYSASFLYSGVPSRFSGSRSGTDFTLTISSLQPEDFATYYCQQHYTTPPTFGQGTKVEIKRTVAAPSVFIFPPSDEQLKSGTASVVCLLNNFYPREAKVQWKVDNALQSGNSQESVTEQDSKDSTYSLSSTLTLSKADYEKHKVYACEVTHQGLSSPVTKSFNRGEC

SEQ ID NO: 50 - protein, 450 aa, synthetic construct
  REGION 1..450: note = Trastuzumab Heavy Chain
EVQLVESGGGLVQPGGSLRLSCAASGFNIKDTYIHWVRQAPGKGLEWVARIYPTNGYTRYADSVKGRFTISADTSKNTAYLQMNSLRAEDTAVYYCSRWGGDGFYAMDYWGQGTLVTVSSASTKGPSVFPLAPSSKSTSGGTAALGCLVKDYFPEPVTVSWNSGALTSGVHTFPAVLQSSGLYSLSSVVTVPSSSLGTQTYICNVNHKPSNTKVDKKVEPKSCDKTHTCPPCPAPELLGGPSVFLFPPKPKDTLMISRTPEVTCVVVDVSHEDPEVKFNWYVDGVEVHNAKTKPREEQYNSTYRVVSVLTVLHQDWLNGKEYKCKVSNKALPAPIEKTISKAKGQPREPQVYTLPPSREEMTKNQVSLTCLVKGFYPSDIAVEWESNGQPENNYKTTPPVLDSDGSFFLYSKLTVDKSRWQQGNVFSCSVMHEALHNHYTQKSLSLSPGK

SEQ ID NO: 51 - protein, 450 aa, synthetic construct
  REGION 1..450: note = Modified HER2 antibody Heavy Chain
EVQLVESGGGLVQPGGSLRLSCAASGFNIKDTYIHWVRQAPGKGLEWVARIYPTNGYTRYADSVKGRFTISADTSKNTAYLQMNSLRAEDTAVYYCSRWGGDGFYAMDYWGQGTLVTVSSASTKGPSVFPLAPSSKSTSGGTAALGCLVKDYFPEPVTVSWNSGALTSGVHTFPAVLQSSGLYSLSSVVTVPSSSLGTQTYICNVNHKPSNTKVDKKVEPKSCDKTHTCPPCPAPEAAGGPSVFLFPPKPKDTLMISRTPEVTCVVVDVSHEDPEVKFNWYVDGVEVHNAKTKPREEQYNSTYRVVSVLTVLHQDWLNGKEYKCKVSNKALPAPIEKTISKAKGQPREPQVYTLPPSREEMTKNQVSLTCLVKGFYPSDIAVEWESNGQPENNYKTTPPVLDSDGSFFLYSKLTVDKSRWQQGNVFSCSVMHEALHNHYTQKSLSLSPGK

SEQ ID NO: 52 - protein, 214 aa, synthetic construct
  REGION 1..214: note = Pertuzumab Light Chain
DIQMTQSPSSLSASVGDRVTITCKASQDVSIGVAWYQQKPGKAPKLLIYSASYRYTGVPSRFSGSGSGTDFTLTISSLQPEDFATYYCQQYYIYPYTFGQGTKVEIKRTVAAPSVFIFPPSDEQLKSGTASVVCLLNNFYPREAKVQWKVDNALQSGNSQESVTEQDSKDSTYSLSSTLTLSKADYEKHKVYACEVTHQGLSSPVTKSFNRGEC

SEQ ID NO: 53 - protein, 449 aa, synthetic construct
  REGION 1..449: note = Pertuzumab Heavy Chain
EVQLVESGGGLVQPGGSLRLSCAASGFTFTDYTMDWVRQAPGKGLEWVADVNPNSGGSIYNQRFKGRFTLSVDRSKNTLYLQMNSLRAEDTAVYYCARNLGPSFYFDYWGQGTLVTVSSASTKGPSVFPLAPSSKSTSGGTAALGCLVKDYFPEPVTVSWNSGALTSGVHTFPAVLQSSGLYSLSSVVTVPSSSLGTQTYICNVNHKPSNTKVDKKVEPKSCDKTHTCPPCPAPELLGGPSVFLFPPKPKDTLMISRTPEVTCVVVDVSHEDPEVKFNWYVDGVEVHNAKTKPREEQYNSTYRVVSVLTVLHQDWLNGKEYKCKVSNKALPAPIEKTISKAKGQPREPQVYTLPPSREEMTKNQVSLTCLVKGFYPSDIAVEWESNGQPENNYKTTPPVLDSDGSFFLYSKLTVDKSRWQQGNVFSCSVMHEALHNHYTQKSLSLSPGK

SEQ ID NO: 54 - protein, 449 aa, synthetic construct
  REGION 1..449: note = Modified HER2 Antibody 2 Heavy Chain
EVQLVESGGGLVQPGGSLRLSCAASGFTFTDYTMDWVRQAPGKGLEWVADVNPNSGGSIYNQRFKGRFTLSVDRSKNTLYLQMNSLRAEDTAVYYCARNLGPSFYFDYWGQGTLVTVSSASTKGPSVFPLAPSSKSTSGGTAALGCLVKDYFPEPVTVSWNSGALTSGVHTFPAVLQSSGLYSLSSVVTVPSSSLGTQTYICNVNHKPSNTKVDKRVEPKSCDKTHTCPPCPAPEAAGGPSVFLFPPKPKDTLMISRTPEVTCVVVDVSHEDPEVKFNWYVDGVEVHNAKTKPREEQYNSTYRVVSVLTVLHQDWLNGKEYKCKVSNKALPAPIEKTISKAKGQPREPQVYTLPPSREEMTKNQVSLTCLVKGFYPSDIAVEWESNGQPENNYKTTPPVLDSDGSFFLYSKLTVDKSRWQQGNVFSCSVMHEALHNHYTQKSLSLSPGK

SEQ ID NO: 55 - protein, 213 aa, synthetic construct
  REGION 1..213: note = Anti-CDH6 Antibody Light Chain
DIQMTQSPSSLSASVGDRVTITCKASQNIYKNLAWYQQKPGKAPKLLIYDANTLQTGVPSRFSGSGSGSDFTLTISSLQPEDFATYFCQQYYSGWAFGQGTKVEIKRTVAAPSVFIFPPSDEQLKSGTASVVCLLNNFYPREAKVQWKVDNALQSGNSQESVTEQDSKDSTYSLSSTLTLSKADYEKHKVYACEVTHQGLSSPVTKSFNRGEC

SEQ ID NO: 56 - protein, 452 aa, synthetic construct
  REGION 1..452: note = Anti-CDH6 Antibody Heavy Chain
EVQLVQSGAEVKKPGASVKVSCKASGYTFTRNFMHWVRQAPGQGLEWMGWIYPGDGETEYAQKFQGRVTITADTSTSTAYMELSSLRSEDTAVYYCARGVYGGFAGGYFDFWGQGTLVTVSSASTKGPSVFPLAPSSKSTSGGTAALGCLVKDYFPEPVTVSWNSGALTSGVHTFPAVLQSSGLYSLSSVVTVPSSSLGTQTYICNVNHKPSNTKVDKRVEPKSCDKTHTCPPCPAPEAAGGPSVFLFPPKPKDTLMISRTPEVTCVVVDVSHEDPEVKFNWYVDGVEVHNAKTKPREEQYNSTYRVVSVLTVLHQDWLNGKEYKCKVSNKALGAPIEKTISKAKGQPREPQVYTLPPSREEMTKNQVSLTCLVKGFYPSDIAVEWESNGQPENNYKTTPPVLDSDGSFFLYSKLTVDKSRWQQGNVFSCSVMHEALHNHYTQKSLSLSPGK

SEQ ID NO: 57 - protein, 6 aa, synthetic construct
  REGION 1..6: note = Pertuzumab CDRL1
QDVSIG

SEQ ID NO: 58 - skipped

SEQ ID NO: 59 - protein, 9 aa, synthetic construct
  REGION 1..9: note = Pertuzumab CDRL3
QQYYIYPYT

SEQ ID NO: 60 - protein, 8 aa, synthetic construct
  REGION 1..8: note = Pertuzumab CDRH1
GFTFTDYT

SEQ ID NO: 61 - protein, 8 aa, synthetic construct
  REGION 1..8: note = Pertuzumab CDRH2
VNPNSGGS

SEQ ID NO: 62 - protein, 12 aa, synthetic construct
  REGION 1..12: note = Pertuzumab CDRH3
ARNLGPSFYFDY

SEQ ID NO: 63 - protein, 11 aa, synthetic construct
  REGION 1..11: note = Anti-CDH6 Antibody CDRL1
KASQNIYKNLA

SEQ ID NO: 64 - protein, 7 aa, synthetic construct
  REGION 1..7: note = Anti-CDH6 Antibody CDRL2
DANTLQT

SEQ ID NO: 65 - protein, 8 aa, synthetic construct
  REGION 1..8: note = Anti-CDH6 Antibody CDRL3
QQYYSGWA

SEQ ID NO: 66 - protein, 5 aa, synthetic construct
  REGION 1..5: note = Anti-CDH6 Antibody CDRH1
RNFMH

SEQ ID NO: 67 - protein, 17 aa, synthetic construct
  REGION 1..17: note = Anti-CDH6 Antibody CDRH2
WIYPGDGETEYAQKFQG

SEQ ID NO: 68 - protein, 13 aa, synthetic construct
  REGION 1..13: note = Anti-CDH6 Antibody CDRH3
GVYGGFAGGYFDF

SEQ ID NO: 69 - protein, 995 aa, Streptococcus pyogenes
MDKHLLVKRTLGCVCAATLMGAALATHHDSLNTVKAEEKTVQVQKGLPSIDSLHYLSENSKKEFKEELSKAGQESQKVKEILAKAQQADKQAQELAKMKIPEKIPMKPLHGPLYGGYFRTWHDKTSDPTEKDKVNSMGELPKEVDLAFIFHDWTKDYSLFWKELATKHVPKLNKQGTRVIRTIPWRFLAGGDNSGIAEDTSKYPNTPEGNKALAKAIVDEYVYKYNLDGLDVDVEHDSIPKVDKKEDTAGVERSIQVFEEIGKLIGPKGVDKSRLFIMDSTYMADKNPLIERGAPYINLLLVQVYGSQGEKGGWEPVSNRPEKTMEERWQGYSKYIRPEQYMIGFSFYEENAQEGNLWYDINSRKDEDKANGINTDITGTRAERYARWQPKTGGVKGGIFSYAIDRDGVAHQPKKYAKQKEFKDATDNIFHSDYSVSKALKTVMLKDKSYDLIDEKDFPDKALREAVMAQVGTRKGDLERFNGTLRLDNPAIQSLEGLNKFKKLAQLDLIGLSRITKLDRSVLPANMKPGKDTLETVLETYKKDNKEEPATIPPVSLKVSGLTGLKELDLSGFDRETLAGLDAATLTSLEKVDISGNKLDLAPGTENRQIFDTMLSTISNHVGSNEQTVKFDKQKPTGHYPDTYGKTSLRLPVANEKVDLQSQLLFGTVTNQGTLINSEADYKAYQNHKIAGRSFVDSNYHYNNFKVSYENYTVKVTDSTLGTTTDKTLATDKEETYKVDFFSPADKTKAVHTAKVIVGDEKTMMVNLAEGATVIGGSADPVNARKVFDGQLGSETDNISLGWDSKQSIIFKLKEDGLIKHWRFFNDSARNPETTNKPIQEASLQIFNIKDYNLDNLLENPNKFDDEKYWITVDTYSAQGERATAFSNTLNNITSKYWRVVFDTKGDRYSSPVVPELQILGYPLPNADTIMKTVTTAKELSQQKDKFSQKMLDELKIKEMALETSLNSKIFDVTAINANAGVLKDCIEKRQLLKK

SEQ ID NO: 70 - protein, 843 aa, Streptococcus pyogenes
MDKHLLVKRTLGCVCAATLMGAALATHHDSLNTVKAEEKTVQTGKTDQQVGAKLVQEIREGKRGPLYAGYFRTWHDRASTGIDGKQQHPENTMAEVPKEVDILFVFHDHTASDSPFWSELKDSYVHKLHQQGTALVQTIGVNELNGRTGLSKDYPDTPEGNKALAAAIVKAFVTDRGVDGLDIDIEHEFTNKRTPEEDARALNVFKEIAQLIGKNGSDKSKLLIMDTTLSVENNPIFKGIAEDLDYLLRQYYGSQGGEAEVDTINSDWNQYQNYIDASQFMIGFSFFEESASKGNLWFDVNEYDPNNPEKGKDIEGTRAKKYAEWQPSTGGLKAGIFSYAIDRDGVAHVPSTYKNRTSTNLQRHEVDNISHTDYTVSRKLKTLMTEDKRYDVIDQKDIPDPALREQIIQQVGQYKGDLERYNKTLVLTGDKIQNLKGLEKLSKLQKLELRQLSNVKEITPELLPESMKKDAELVMVGMTGLEKLNLSGLNRQTLDGIDVNSITHLTSFDISHNSLDLSEKSEDRKLLMTLMEQVSNHQKITVKNTAFENQKPKGYYPQTYDTKEGHYDVDNAEHDILTDFVFGTVTKRNTFIGDEEAFAIYKEGAVDGRQYVSKDYTYEAFRKDYKGYKVHLTASNLGETVTSKVTATTDETYLVDVSDGEKVVHHMKLNIGSGAIMMENLAKGAKVIGTSGDFEQAKKIFDGEKSDRFFTWGQTNWIAFDLGEINLAKEWRLFNAETNTEIKTDSSLNVAKGRLQILKDTTIDLEKMDIKNRKEYLSNDENWTDVAQMDDAKAIFNSKLSNVLSRYWRFCVDGGASSYYPQYTELQILGQRLSNDVANTLKD

SEQ ID NO: 71 - protein, 928 aa, Streptococcus iniae
MNKRLLVKRTFGCVCAAAILGVAPLSHPTIVEAREELKMPNGLEQSIADVEAKIDALTYLSKNSKDEFKHSMYEIPSNREHKPVSPKQALQNAKKADAQAERLAKMTIPKKEELKALEGPLYGGYFRTWQDKTSDPTETNKVNSFGELPKEVDLAFVFHDYTKDYSLFWEELATKQVPKLNKQGTRVIRTIPWRFLSGADHSDISADKEKFPNTEAGNKALAKAIVDEYVYKYNLDGLDIDIERDSVPKVNDKEDPEALARTVEVFKEIGKLIGANGADKSRLLIMDTTYTAEENPLIKETAQYLNLLLVQVYGFSGENGNYLHHKNILDETSSMEGRWQGYSKYIRPEQYMVGFSFYEEKDFNNRWKDINEEDPSDPHIGEKIQGTRAERYAKWQPKTGGLKGGLFSYAIDRDGVAQPKQKTEHPELDKIVKSEYKVSKALKKLMMTDDQYQPIDQSDFPDKALRESIIKQVGTRRGDLERFKGTLRLDNPEIKDLTGLNKLKRVAKLELINLPKITKIDKDDLPQNLKPLTDNQKSNLEIKGTYDDSKLYKDIPAFDLVISGLSGLESLDISGHQRDTLSGIDASTLPSLKAINISDNHFDLAQGTENRHILDTILATLAKNGASTASFDKQKPKGLYPESYSTAPLHLQVGQGKINVIDDLIFGTRTNQNTLINTENDFEAYKEQTIQGKPFIAPDYLYDNFKVSYKEYSASIVDSTLAETTDKTIDTAKAETYQVTVSNKDGKTVHSVKVIVGDEKPMMVNLAQDAKIIGTDNMTQSAKVFDGQKDQFLLSWNKDSSVIFELKTPGTAKHWRFFDDGKNDSVTLSVFKGDASNFETEKDKAENWVEITKDSRKNDDKVFSSPLEVDNAKYLKVTIKKEAKYIYFNELQILGYPGVVAKKTADDLRPTEADKSDDKSDKNDTEAK

SEQ ID NO: 72 - protein, 744 aa, Mucor hiemalis
MPSLQLQPDDKLAPVSFALKSMNELRDWTPDEKIKFNVSSVALQPRVKNALKPQLLLTHDMAGGYKEDKNIQGNNYKDIYNIQYWHLADTFVYFSHERVSIPPVNWTNACHRNGVKCLGTFLVEGNNQMHEMEALLHGPPLLNNTDDPMRLWSPYYADQLVAIAKHYGFDGWLFNIECEFFPFPTNPKFKAEELAKFLHYFKEKLHNEIPGSQLIWYDSMTNEGEIHWQNQLTWKNELFFKNTDGIFLNYWWKKEYPEMARRVAEGIGRSGLEVYFGTDVWGRHTYGGGGFKSYKGVKTAYSAMTSSALFGMAWTYEHFEKSEFEKMDRLFWCGGKYSDYPPPPPKNPDDEKEVESDDSEDELMYGHKKGIADTVESIPVPGTDWFVTNFDRGFGNRFYYRGKRLLSQPWSHLSHQAILPNKSYRNPEIYPTDQNIKITSSLDCDHGAFLGGTSLIIKGQRFNHRESHDVETEISIPLYKLSLDASKGCSLRYIYRTLLMKDVKLTVACHFSLKTNDSVNFFKVWQPDENFSFEYDDGMRATVTTENSTESRCFLLRTTEEDTGENDWITKTINVPAVPEGSQLYITRLEVSVVLDTAGLVGLVNQVIACLGYISIIPTINSGIKTDSSRIIQDLFWKDQKYTKIGKESLDDIAQEEVHRYYGTLNWENTANVVNAWEEIDYYNVFYKESDDSATRIFLGTAFCNQFRVSGLDIILSKLPKIVIEAVNKEGYISSSGSIDLSLN

SEQ ID NO: 73 - protein, 696 aa, Rhizomucor pusillus [sequence omitted]

SEQ ID NO: 74 - protein, 787 aa, Coprinopsis cinerea
MPIAGKKFHPRALPEFWRTFREMDEWRATQTGPQARPAEGILKYVPRKIRPADIAGKGRLLVSHDYKGGYVEDPFSKSYSFNWWFSTDSFNYFAHHRITIPPPEWINAAHRQGVPILGTIIFEGGSDEDILRMVIGKTPGSTSNFHAERNAEYTVPVSSYYAELFADLAVERGFDGWLLNVEIGLQGGSEQARGLAAWVALLQQEVLKKVGPHGLVIWYDSVTVRGDLWWQDRLNAFNLPFFLNSSGIFTNYWWYNDAPQKQIDFLSRVDPNLTGQTAEPHQYNLQKTIQDIYIGVDVWGRGSHGGGGFGAYKAIEHADPKGLGFSVALFAQGWTWETEEEKPGWNWAQFWDYDSKLWVGPPGVVEAPDHTVKPGEYPCVHGPFQPISSFFLTYPPPDPLDLPFYTNFCPGIGDAWFVEGKEVFRSETGWTDMDKQTTVGDLVWPRPKIYDLPSQNASQATLNAAFNFNDAWNGGNSLQINLTVPGGATTYGAYWVPIQTFTFSSRRQYEASIVYKPGLSGKTRFDAKYEVGIRTITGEDQGKIISNTTTEVGNGWRKVHILFEIETPVEGGSIIVPSSIGLVIAVSNVSTTEQFEFPFLVGQITIHPHLPDRYKEFKPALLWLLFTPSAGTNSLDGTLTWDVVAAIERPPPVEINNPDDAQIPWNLQPTKQEWFPDFLYFNVYVLELLDGGGQGPPQWIGTTGYDGEKKRFFIYDESLPPTSGLRRFTFQIEGVLETGESTHWYDAPAAPSATAGGEQKRTRRTSLKSVLSPLRRKKSKGDISVAK

SEQ ID NO: 75 - protein, 772 aa, Ogataea minuta
MAQSQLLGGAVRPVFFDKLEELRRWHTQSANLSRESELDSLNVATEPFSSYERAQTGSGSRSSEPVPGDKEDPPIKLMVCHDFKGGYQDYEDAQPLGYFPHPTGSRYFLQYPQLIDQFVYFSHHRVTVPPVNWINFCHRNGIKCFGTVIFEGNASKDFEELDRLVSRDEKGDFVFVDALIKLAAHYGFDGYLLNIETTFSNTKIAADLEPFAEQLKSGLHCLDSKNELIWYDSYVFPANKVSYTNGVTESNYNFFSLSDAFFSNYWWNIKNLQENIKNVGVLGVQKKIYVGYDVWGRGTLVGKGGFDSSLACKMIAKFKSNVALFAPAWTYESLGPKDFNQNDARFWIGLFENESSISSTVPPHSSAVYKINESSFIFYTNFSSGEGNRFFSKGSEVYRKNWVNGSLQFDLPIDLHRKDKNGLQWALDKSDAFHGGACLEIKYSEIKDENGYQIFNNQMVSDFTLFNFTKECHFPTVNVKVTYKLNHKTKSTFKIKIKYIIERRFRSVQTVRTGYLTIPLLSTSGKWFTVEESFQINLQTSHEYIVLESAHVTYDEDRSADSFFRSYIVEDSAITSVIDNEEYEKLINSEIYNDDEDEDWILVPSDVSISSSESQSNDSKTQYLGRKLFGNKSTPKTRTLEGTAPLLRIGEFAIISANNYPSSNFLAVTSVKSIESSRLEGDSLVLLNWQVGEGHQKGVCYYIIYVNGAVVGLSVAPKFIYQDTELASENSASARSNYKKSGLGSSSDRKSKVRVDSVDKLGNVFTGSEVWV

SEQ ID NO: 76 - protein, 1067 aa, Streptococcus dysgalactiae
MDKRLLVKRTLGCVCSATLMGTILGTHHDSLISVKAEEKITQVSQTSTSIDDLHYLSENSKKEFKEELSKEKVPEKVKEILSKAQQANKQAQELAEMKVPDKIPMKPLNGPLYGGYFRTWHDKTSDPLEKDKVNSMGELPKEVDLAFVFHDWTKDYSLFWKELATKHVPKLNKQGTRVIRTIPWRFLAGGDNSGIAEDASKYPNTPEGNKALAKAIVDEYVYKYNLDGLDVDIEHDSIPKVNGEASDENLKRSIDVFEEIGKLIGPKGADKSRLFIMDSTYMADKNPLIERGAPYIDLLLVQVYGSQGEQGEFQNDTKSVTKTPEERWQGYSKYIRPEQYMIGFSFYEEKAGSGNLWYDINARKDEDTANGINDDITGTRAERYARWQPKTGGVKGGIFSYAIDRDGVAHQPKQIAEKDKQSVKNNRPLISEITDNIFHSNYSVSKTLKTVMLKDKAYDLIDEKDFPDKALREAVMAQVGTRKGDLERFNGTLRLDNPAIQSLEGLNKFKKLAQLDLIGLSRIIKLDQSVLPANMKPGKDPLETVLETYKKNGKEEPAIIPPVSLTVSGLTGLKELDLSGFDRETLAGIDAATLTSLEKVDISDNKLDLAPKTENRQIFDVMLSTVNNNAGISEQSIKFDNQKPAGNYPQTYGATNLQLPVRQEKIDLQHQLLFGTITNQGTLINSEADYKTYRNQKIAGRNFVDPDYPYNNFKVSHDNYTVKVTDSTLGTTTDKMLATDKEETYKVDFFSPTDKTKAVHTAKVIVGDEKTMMVNLAEGATVIKSENDENAQKVFNGIMEYNPLSFNNKSSIIFEIKDPSLAKYWRLFNDSSKDKKDYIKEAKLEVFTGQLNAEADVKTILEKPDNWVTVSTYSGEEKVFSHSLDNISAKYWRVTVDNKKDQYGYVSLPELQILGYPLPNADTIMKTVTVAKELSQQKDKFPQQLLDESTAKEAVVEASLNSKLFDTGVINTNVEALKNVVDECLAYEKNKETAFKATEDYRAAVNGVKAESVTVEEMAQLKDLIGKAAHLNSKIDAKLADREYDKDLLGLIGELTNITRTVKSFVK

SEQ ID NO: 77 - protein, 1011 aa, Streptococcus equi
MEKQVLVKKTLKCVCAAALMVAILAAQHDSLIRVKAEDKLVQTSPSVSAIDALHYLSENSKKEFKEELSKVEKAQPEKLKEIVSKAQQADKQAKTLAEMKVPEKIPMKPLKGPLYGGYFRTWHDKTSDPAEKDKVNSMGELPKEVDLAFVFHDWTKDYSLFWQELATKHVPTLNKQGTRVIRTIPWRFLAGGDHSGIAEDAQKYPNTPEGNKALAKAIVDEYVYKYNLDGLDVDIERDSIPKVNKEESKEGIERSIQVFEEIGKLIGPKGADKSRLFIMDSTYMADKNPLIERGAPYIDLLLVQVYGTQGEKGGFDNANHKAVDTMEERWESYSKYIRPEQYMVGFSFYEEKANSGNLWYDVNVEDDTNPNIGSEIKGTRAERYAKWQPKTGGVKGGIFSYGIDRDGVAHPKKNGPKTPDLDKIVKSDYKVSKALKKVMENDKSYELIDQKDFPDKALREAVIAQVGSRRGNLERFNGTLRLDNPDIKSLEGLNKLKKLAKLELIGLSQITKLDSSVLPENIKPTKDTLVSVLETYKNDDRKEEAKAIPQVALTISGLTGLKELNLAGFDRDSLAGIDAASLTSLEKVDLSSNKLDLAAGTENRQILDTMLATVTKHGGVSEKTFVFDHQKPTGLYPDTYGTKSLQLPVANDTIDLQAKLLFGTVTNQGTLINSEADYKAYQEQEIAGHRFVDSSYDYKAFAVTYKDYKIKVTDSTLGVTDHKDLSTSKEETYKVEFFSPINSTKPVHEAKIVVGEEKTMMVNLAEGATIIGGDADPTNAKKVFDGLLNNDTTTLSTSNKASIIFELKEPGLVKHWRFFNDSKISKADYIKEAKLEAFVGHLEDSSKVKDSLEKSTEWVTVSDYSGEAQEFSQPLNNIGAKYWRITIDNKKSQYGYVSLPELQIIGHRLPEAATVMTTMAAAEELSQQKDKFSQEQLKELEVKVAALKAALDNKMFNADTINASFADVKAYIDKLLADAAGKKTLGKATKEAQPVATDAKEKAESENPKAD

SEQ ID NO: 78 - protein, 1018 aa, Streptococcus equi
MEKQVLVKKTLKCVCAAALMVAILAAQHDSLIRVKAEDKVVQTSPSVSAIDDLHYLSENSKKEFKEGLSKAGEVPEKLKDILSKAQQADKQAKVLAEMKVPEKIAMKPLKGPLYGGYFRTWHDKTSDPAEKDKVNSMGELPKEVDLAFVFHDWTKDYSFFWQELATKHVPTLNKQGTRVIRTIPWRFLAGGDHSGIAEDTQKYPNTPEGNKALAKAIVDEYVYKYNLDGLDVDIERDSIPKVNGKESNENIQRSIAVFEEIGKLIGPKGADKSRLFIMDSTYMADKNPLIERGAQYIDLLLVQVYGTQGEKGDWDPVARKPEKTMEERWESYSKYIRPEQYMVGFSFYEENAGSGNLWYDINERKDDHNPLNSEIAGTRAERYAKWQPKTGGVKGGIFSYAIDRDGVAHQPKKVSDDEKRTNKAIKDITDGIVKSDYKVSKALKKVMENDKSYELIDQKDFPDKALREAVIAQVGSRRGDLERFNGTLRLDNPDIKSLEGLNKLKKLAKLELIGLSQITKLDSLVLPANAKPTKDTLANVLEAYDSAKKEETKAIPQVALTISGLTGLKELNLAGFDRDSLAGIDAASLTSLEKVDLSSNKLDLAAGTENRQILDTMLATVTKHGGVSEKTFVFDHQKPTGLYPDTYGTKSLQLPVANDTIDLQAKLLFGTVTNQGTLINSEADYKAYQEQEIAGHRFVDSSYDYKAFAVTYKDYKIKVTDSTLGVTDHKDLSTSKEETYKVEFFSPTNSTKPVHEAKVVVGAEKTMMVNLAEGATVIGGDADPTNAKKVFDGLLNNDTTILSTSNKASIIFELKEPGLVKYWRFFNDSKISKADCIKEAKLEAFVGHLEAGSKVKDSLEKSSKWVTVSDYSGEDQEFSQPLNNIGAKYWRITVDTKGGRYNWPSLPELQIIGYQLPAADLVMAMLATAEELSQQKDKFSQEQLKELEVKIAALKAALDSKMFNADAINASTADLKAYVDKLLADRTDQEKVAKAAKVEQPVATDIKENTEPENPKTD

SEQ ID NO: 79 - protein, 1629 aa, synthetic construct
MREELKMPNGLEQSIADVEAKIDALTYLSKNSKDEFKHSMYEIPSNREHKPVSPKQALQNAKKADAQAERLAKMTIPKKEELKALEGPLYGGYFRTWQDKTSDPTETNKVNSFGELPKEVDLAFVFHDYTKDYSLFWEELATKQVPKLNKQGTRVIRTIPWRFLSGADHSDISADKEKFPNTEAGNKALAKAIVDEYVYKYNLDGLDIQIERDSVPKVNDKEDPEALARTVEVFKEIGKLIGANGADKSRLLIMDTTYTAEENPLIKETAQYLNLLLVLVYGFSGENGNYLHHKNILDETSSMEGRWQGYSKYIRPEQYMVGFSFYEEKDFNNRWKDINEEDPSDPHIGEKIQGTRAERYAKWQPKTGGLKGGLFSYAIDRDGVAQPKQKTEHPELDKIVKSEYKVSKALKKLMMTDDQYQPIDQSDFPDKALRESIIKQVGTRRGDLERFKGTLRLDNPEIKDLTGLNKLKRVAKLELINLPKITKIDKDDLPQNLKPLTDNQKSNLEIKGTYDDSKLYKDIPAFDLVISGLSGLESLDISGHQRDTLSGIDASTLPSLKAINISDNHFDLAQGTENRHILDTILATLAKNGASTASFDKQKPKGLYPESYSTAPLHLQVGQGKINVIDDLIFGTRTNQNTLINTENDFEAYKEQTIQGKPFIAPDYLYDNFKVSYKEYSASIVDSTLAETTDKTIDTAKAETYQVTVSNKDGKTVHSVKVIVGDEKPMMVNLAQDAKIIGTDNMTQSAKVFDGQKDQFLLSWNKDSSVIFELKTPGTAKHWRFFDDGKNDSVTLSVFKGDASNFETEKDKAENWVEITKDSRKNDDKVFSSPLEVDNAKYLKVTIKKEAKYIYFNELQILGYPGVVAKKTADDLRPTEADKSDDKSDKNDTEAKGGGGSGGGGSGGGGSHHHHHHEFGGGGSGGGGSGGGGSPSLELQQAADTRLFESMPLQTMNELGSWEPSNASRANIATIPLHQRSNLDPAEPRLIVTHDMAGGYKEDSNIQGNTYDTIYSCQYWQYVDTFIYFSHHRVTIPPVNWINACHRNGVKTLGTFIVEGAAGMFALERFVYGPEPGQRNSWSPYYADKLVDIAEFYGFDGWLLVIESDFFPLYRNPSLKAIHLAKLLRYLKNAMHARVPGSEIIWYDSMTTNGSVQWQNNITPKNSIFFEAADGIFLNYWWNATVPPLALQVAHRLGRQGSDVYFGTDVWGRGTFGGGGFDSYLAVGTARAFKTSSALFGTAWIYEHFGKKDFELMDRLLWLGGDQSEYPAQEGEQNRTVKVTSHLGRHPGIADVSPVRSAPGKTWFATWFDRGYGTGFYYQGKKLLSQPWSHLSHQSIPPNLIARLQREENHGLSYFLADDDAYIGGTSLLIAAEITQERQLPLYQLEYDVTEGCEVQFIYKSPEPDMQGKIDIYLNLQVTDILPDELAFYWQDVTDASSQADATTAMRLYLNENTVIYLKPSRKQELAEGWLLCSVRVPPTYPLGIATIKELGIHVDGKETVLFRLGLLTIIPLGDAPSALSRITQVQLQRDEDIHSKCPSSSCELWATLSWMMEHNSKEDWDQVDHYMIFFKNVDSKAEPIFLGTSFSTEYRISGLEIKKHGNSIEIWAVNRLGTVIARQDIDIQ

SEQ ID NO: 80 - protein, 1629 aa, synthetic construct
MPSLELQQAADTRLFESMPLQTMNELGSWEPSNASRANIATIPLHQRSNLDPAEPRLIVTHDMAGGYKEDSNIQGNTYDTIYSCQYWQYVDTFIYFSHHRVTIPPVNWINACHRNGVKTLGTFIVEGAAGMFALERFVYGPEPGQRNSWSPYYADKLVDIAEFYGFDGWLLVIESDFFPLYRNPSLKAIHLAKLLRYLKNAMHARVPGSEIIWYDSMTTNGSVQWQNNITPKNSIFFEAADGIFLNYWWNATVPPLALQVAHRLGRQGSDVYFGTDVWGRGTFGGGGFDSYLAVGTARAFKTSSALFGTAWIYEHFGKKDFELMDRLLWLGGDQSEYPAQEGEQNRTVKVTSHLGRHPGIADVSPVRSAPGKTWFATWFDRGYGTGFYYQGKKLLSQPWSHLSHQSIPPNLIARLQREENHGLSYFLADDDAYIGGTSLLIAAEITQERQLPLYQLEYDVTEGCEVQFIYKSPEPDMQGKIDIYLNLQVTDILPDELAFYWQDVTDASSQADATTAMRLYLNENTVIYLKPSRKQELAEGWLLCSVRVPPTYPLGIATIKELGIHVDGKETVLFRLGLLTIIPLGDAPSALSRITQVQLQRDEDIHSKCPSSSCELWATLSWMMEHNSKEDWDQVDHYMIFFKNVDSKAEPIFLGTSFSTEYRISGLEIKKHGNSIEIWAVNRLGTVIARQDIDIQGGGGSGGGGSGGGGSHHHHHHEFGGGGSGGGGSGGGGSREELKMPNGLEQSIADVEAKIDALTYLSKNSKDEFKHSMYEIPSNREHKPVSPKQALQNAKKADAQAERLAKMTIPKKEELKALEGPLYGGYFRTWQDKTSDPTETNKVNSFGELPKEVDLAFVFHDYTKDYSLFWEELATKQVPKLNKQGTRVIRTIPWRFLSGADHSDISADKEKFPNTEAGNKALAKAIVDEYVYKYNLDGLDIQIERDSVPKVNDKEDPEALARTVEVFKEIGKLIGANGADKSRLLIMDTTYTAEENPLIKETAQYLNLLLVLVYGFSGENGNYLHHKNILDETSSMEGRWQGYSKYIRPEQYMVGFSFYEEKDFNNRWKDINEEDPSDPHIGEKIQGTRAERYAKWQPKTGGLKGGLFSYAIDRDGVAQPKQKTEHPELDKIVKSEYKVSKALKKLMMTDDQYQPIDQSDFPDKALRESIIKQVGTRRGDLERFKGTLRLDNPEIKDLTGLNKLKRVAKLELINLPKITKIDKDDLPQNLKPLTDNQKSNLEIKGTYDDSKLYKDIPAFDLVISGLSGLESLDISGHQRDTLSGIDASTLPSLKAINISDNHFDLAQGTENRHILDTILATLAKNGASTASFDKQKPKGLYPESYSTAPLHLQVGQGKINVIDDLIFGTRTNQNTLINTENDFEAYKEQTIQGKPFIAPDYLYDNFKVSYKEYSASIVDSTLAETTDKTIDTAKAETYQVTVSNKDGKTVHSVKVIVGDEKPMMVNLAQDAKIIGTDNMTQSAKVFDGQKDQFLLSWNKDSSVIFELKTPGTAKHWRFFDDGKNDSVTLSVFKGDASNFETEKDKAENWVEITKDSRKNDDKVFSSPLEVDNAKYLKVTIKKEAKYIYFNELQILGYPGVVAKKTADDLRPTEADKSDDKSDKNDTEAK

SEQ ID NO: 81 - protein, 1629 aa, synthetic construct
MPSLELQQAADTRLFESMPLQTMNELGSWEPSNASRANIATIPLHQRSNLDPAEPRLIVTHDMAGGYKEDSNIQGNTYDTIYSCQYWQYVDTFIYFSHHRVTIPPVNWINACHRNGVKTLGTFIVEGAAGMFALERFVYGPEPGQRNSWSPYYADKLVDIAEFYGFDGWLLHIESDFFPLYRNPSLKAIHLAKLLRYLKNAMHARVPGSEIIWYDSMTTNGSVQWQNNITPKNSIFFEAADGIFLNYWWNATVPPLALQVAHRLGRQGSDVYFGTDVWGRGTFGGGGFDSYLAVGTARAFKTSSALFGTAWIYEHFGKKDFELMDRLLWLGGDQSEYPAQEGEQNRTVKVTSHLGRHPGIADVSPVRSAPGKTWFATWFDRGYGTGFYYQGKKLLSQPWSHLSHQSIPPNLIARLQREENHGLSYFLADDDAYIGGTSLLIAAEITQERQLPLYQLEYDVTEGCEVQFIYKSPEPDMQGKIDIYLNLQVTDILPDELAFYWQDVTDASSQADATTAMRLYLNENTVIYLKPSRKQELAEGWLLCSVRVPPTYPLGIATIKELGIHVDGKETVLFRLGLLTIIPLGDAPSALSRITQVQLQRDEDIHSKCPSSSCELWATLSWMMEHNSKEDWDQVDHYMIFFKNVDSKAEPIFLGTSFSTEYRISGLEIKKHGNSIEIWAVNRLGTVIARQDIDIQGGGGSGGGGSGGGGSHHHHHHEFGGGGSGGGGSGGGGSREELKMPNGLEQSIADVEAKIDALTYLSKNSKDEFKHSMYEIPSNREHKPVSPKQALQNAKKADAQAERLAKMTIPKKEELKALEGPLYGGYFRTWQDKTSDPTETNKVNSFGELPKEVDLAFVFHDYTKDYSLFWEELATKQVPKLNKQGTRVIRTIPWRFLSGADHSDISADKEKFPNTEAGNKALAKAIVDEYVYKYNLDGLDIMIERDSVPKVNDKEDPEALARTVEVFKEIGKLIGANGADKSRLLIMDTTYTAEENPLIKETAQYLNLLLVLVYGFSGENGNYLHHKNILDETSSMEGRWQGYSKYIRPEQYMVGFSFYEEKDFNNRWKDINEEDPSDPHIGEKIQGTRAERYAKWQPKTGGLKGGLFSYAIDRDGVAQPKQKTEHPELDKIVKSEYKVSKALKKLMMTDDQYQPIDQSDFPDKALRESIIKQVGTRRGDLERFKGTLRLDNPEIKDLTGLNKLKRVAKLELINLPKITKIDKDDLPQNLKPLTDNQKSNLEIKGTYDDSKLYKDIPAFDLVISGLSGLESLDISGHQRDTLSGIDASTLPSLKAINISDNHFDLAQGTENRHILDTILATLAKNGASTASFDKQKPKGLYPESYSTAPLHLQVGQGKINVIDDLIFGTRTNQNTLINTENDFEAYKEQTIQGKPFIAPDYLYDNFKVSYKEYSASIVDSTLAETTDKTIDTAKAETYQVTVSNKDGKTVHSVKVIVGDEKPMMVNLAQDAKIIGTDNMTQSAKVFDGQKDQFLLSWNKDSSVIFELKTPGTAKHWRFFDDGKNDSVTLSVFKGDASNFETEKDKAENWVEITKDSRKNDDKVFSSPLEVDNAKYLKVTIKKEAKYIYFNELQILGYPGVVAKKTADDLRPTEADKSDDKSDKNDTEAK